European Patent Application EP 4 119 944 A1, published January 18, 2023. Title: Improved pharmacokinetic assays for immunoglobulin single variable domains. Applicant: Ablynx N.V. The sequence listing filed with the application follows.

SEQUENCE LISTING (5 sequences)

SEQ ID NO: 1 - protein, 5 aa, Artificial Sequence
  C-terminal end of ISVD
VTVSS

SEQ ID NO: 2 - protein, 447 aa, Artificial Sequence
  Quencher
HHHHHHDVQLVESGGGLVQPGGSLRLSCAASGRTFNNYAMGWFRQAPGKEREFVAAITRSGVRSGVSAIYGDSVKDRFTISRDNAKNTLYLQMNSLRPEDTAVYYCAASAIGSGALRRFEYDYSGQGTLVTVSSGGGGSGGGGSGGGGSGGGGSGGGGSGGGGSGGGGSEVQLVESGGGLVQPGGSLRLSCAASGRTFNNYAMGWFRQAPGKEREFVAAITRSGVRSGVSAIYGDSVKDRFTISRDNAKNTLYLQMNSLRPEDTAVYYCAASAIGSGALRRFEYDYSGQGTLVTVSSGGGGSGGGGSGGGGSGGGGSGGGGSGGGGSGGGGSEVQLVESGGGLVQPGNSLRLSCAASGFTFSSFGMSWVRQAPGKGLEWVSSISGSGSDTLYADSVKGRFTISRDNAKTTLYLQMNSLRPEDTAVYYCTIGGSLSRSSQGTLVTVSS

SEQ ID NO: 3 - protein, 121 aa, Artificial Sequence
  Quencher
HHHHHHEVQLVESGGDLVQPGNSLRLSCAASGFTFSSFGMSWVRQAPGKGLEWVSSISGSGSDTLYADSVKGRFTISRDNAKTTLYLQMNSLRPEDTAVYYCTIGGSLSRSSQGTLVTVSS

SEQ ID NO: 4 - protein, 115 aa, Artificial Sequence [sequence omitted]

SEQ ID NO: 5 - protein, 270 aa, Artificial Sequence
  Quencher
EVQLVESGGGLVQPGGSLRLSCAASGFTFSSYAMSWVRQAPGKGLEWVSGIKSSGDSTRYAGSVKGRFTISRDNAKNTLYLQMNSLRPEDTAVYYCAKSRVSRTGLYTYDNRGQGTLVTVSSGGGGSGGGGSGGGGSGGGGSEVQLVESGGGLVQPGGSLRLSCAASGRTFNNYAMGWFRQAPGKEREFVAAITRSGVRSGVSAIYGDSVKDRFTISRDNAKNTLYLQMNSLRPEDTAVYYCAASAIGSGALRRFEYDYSGQGTLVTVSS